European Patent Application EP 4 353 258 A1, published April 17, 2024. Title: à Ì \ h Ü ½ Í ¡ Ã Ì ½ ß Ì ã ò g ¬ ¨. Applicant: National University Corporation University of Toyama. The sequence listing filed with the application follows.

SEQUENCE LISTING (118 sequences)

SEQ ID NO: 1 - protein, 118 aa, Mus musculus
QVQLQQPGAELVRPGSSVKLSCKASGYTFISYWMDWVKQRPGQGLEWIGNIFPSDSETHYNQKFRDKATLTVDKSSSTASIHLSSLTSEDSAVYYCGRRDSSGWIDYWGQGTTLTVSS

SEQ ID NO: 2 - protein, 107 aa, Mus musculus
DIQMTQTTSSLSASLGDRVTISCRASQDISNYLNWYQQKPDGTVKLLIYYTSRFHSGVPSRFSGSGSGTDYSLTIHNVEQEDIATYFCQQSSMLPFTFGSGTKLEMK

SEQ ID NO: 3 - protein, 116 aa, Mus musculus
QVQLQQPGAELVRPGSSVKLSCRASGYTFTSYWMDWVKQRPGQGLEWIGNIYPSDGETHYNQDFKDKATLTVDKSSSTAYMQLSSLTSEDSAVYYCARGTTLFDYWGQGTTLTVSS

SEQ ID NO: 4 - protein, 112 aa, Mus musculus
DVLMTQTPLSLPVSLGDQASISCRSSQSIVHINGNTYLEWYLQKPGQSPKLLIYKVSNRFSGVPDRFSGSGSGTDFTLKISRVEAEDLGIYYCFQGSHVPWTFGGGTKLEIK

SEQ ID NO: 5 - protein, 121 aa, Mus musculus
QVQLQQPGAELVKPRASVKLSCRASGYIFISYWMQWVKQRPGQGLEWIGEIDPSDSYINYNQKFKGKASLTVDTSSNTAYMQLSSLTSEDSAVYYCATGDMGDDFYAMDYWGQGTSVTVSS

SEQ ID NO: 6 - protein, 112 aa, Mus musculus
DIVMNQDELSNPVTSGESVSISCRSSKSLLYKDGKTYLNWFLQRPGQSPQLLIYLMSTRASGVSDRFSGSGSGTDFTLEISRVKAEDVGVYYCQQLVEYPFTFGGGTKLEIK

SEQ ID NO: 7 - protein, 115 aa, Mus musculus
QVQLQQPGAELVKPGASVKVSCKASGYTFTTYWMHWVKQRPGQGLEWIGRIHPSDSDSNYNQKFKGKATLTVDKSSSTAYMQLSSLTSEDSAVYYCAIGRGFAYWGQGTLVTVSA

SEQ ID NO: 8 - protein, 111 aa, Mus musculus
DIVLTQSPASLAVSLGQRAAISCRASESVDNYGNSFMHWYQQKPGQPPKLLIYRASNLESGIPARFSGSGSRTDFTLTINPVEADDVATYYCQQGNEDPYTFGGGTKLEIK

SEQ ID NO: 9 - protein, 117 aa, Mus musculus
QVQLQQSGAELVRPGTSVKVSCKASGYAFTNYLIEWVKQRPGQGLEWIGVINPGSGGTNYNEKFKGKATLTADKSSSTAYMQLSSLTSEDSAVYFCARDYGSTFDYWGQGTTLTVSS

SEQ ID NO: 10 - protein, 107 aa, Mus musculus
DIVLTQSPATLSVTPGDSVSLSCRASQSISSNLHWYQQKSHESPRLLINFASQSISGIPSRFSGSGSGTDFTLNINTVETEDFGMYFCQQSNSWPLTFGAGTKLELK

SEQ ID NO: 11 - protein, 120 aa, Mus musculus
QVQLQQSGAELVRPGTSVKVSCKASGYAFTDYLIEWVKQRPGQGLEWIGVINPGRGGTNYNEKFKGKATLTADKSSSTAYMQLSSLTSEDSAVYFCARYYGRSFGYFDVWGTGTTVTVSS

SEQ ID NO: 12 - protein, 107 aa, Mus musculus
DIQMTQSPASQSASLGESVTITCLASQTIGTWLAWYQQKPGKSPQLLIYAATSLADGVPSRFSGSGSGTKFSFKISSLQAEDFVSYYCQQLYSPPLTFGAGTKLELK

SEQ ID NO: 13 - protein, 118 aa, Mus musculus
QVQLQQPGAELVRPGSSVKLSCKASGYTFTSYWMDWVKQRPGQGLEWIGNIYPSDSETHYNQKFKDRATLTVDKSSTTAYMQLSSLTSEDSAVYYCTRRDSSGWIDYWGQGTTLTVSS

SEQ ID NO: 14 - protein, 107 aa, Mus musculus
DIQMTQTTSSLSASLGDRVTISCRASQDISNYLNWYQQKPDGTVKLLIYYTSRLHSGVPSRFSGRGSGTDYSLTISNLEQEDIATYFCQQGNTLPFTFGSGTQLEIK

SEQ ID NO: 15 - protein, 120 aa, Mus musculus
EVQLVESGGGLVQPKGSLKLSCAASGFSFNTYTMNWVRQAPGKGLEWVARIRSKSNNYETYYADSVKDRFTISRDDSESMLYLQMNNLKTEDTAMYYCVSPDSDSWFAYWGQGTLVTVSA

SEQ ID NO: 16 - protein, 107 aa, Mus musculus
DIQMNQSPSSLSASLGDTITIACHASQNINVWLSWYQQKPGNIPKLLIYKASNLHTGVPSRFSGSGSGTGFTLTISSLQPEDIATYYCQQGQSYPLTFGGGTKLEIK

SEQ ID NO: 17 - protein, 118 aa, Mus musculus
QVQLQQPGAELVKPGASVKMSCKASGYTFSTYWITWVKQRPGQGLEWIGDIYPGGDSTNYNEKFKSKATLTEDTSSSTVYMQLSSLTSEHSAVYYCARGITGGYFDYWGQGTTLTVSS

SEQ ID NO: 18 - protein, 107 aa, Mus musculus
DIQMTQTTSSLSASLGDRVTITCRASQDISNYLNWYQRKPDGTVRLLIYYTSGLHSGVPSRFSGSGSGTDYSLTISNLEQEDFATYFCQQGHTLPWTFGGGTNLEIK

SEQ ID NO: 19 - protein, 118 aa, Mus musculus
QVQLKQSGPGLVQTSQSLSITCTVSGFSLSSYGVHWVRQSPGKGLEWLGVIWSGGSTDYNAAFTSRLSISKDNSKSQVFFKMNSLQADDTAMYYCVSFNYGSSSFAYWGQGTLVTVSA

SEQ ID NO: 20 - protein, 107 aa, Mus musculus
DIVMTQSHKFMSTSVGDRVSITCKASQDVRTAVAWYQQKPGQSPKLLIYSASYRYTGVPDRFTGSGSGTDFTFTISSVQAEDLAVYYCQQHYSTPLTFGAGTKLELK

SEQ ID NO: 21 - protein, 119 aa, Mus musculus
QVQLQQPGAELVRPGSSVKLSCKASGYTFTTYWMHWVKQRPIQGLEWIGNIDPSDSETHYNQKFKDKATLTVDKSSSTAYMQLNSLTSEDSAVYYCARGDGYYVYFAYWGQGTTLTVSS

SEQ ID NO: 22 - protein, 108 aa, Mus musculus
EIVLTQSPALMAASPGEKVTITCSVSSSISSSNLHWYQQKSETSPKPWIYATSNLASGVPVRFSGSGSGTSYSLTISSMAAEDAATYFCQQWSSFPLTFGAGTKLELK

SEQ ID NO: 23 - protein, 117 aa, Mus musculus
QVQLKQSGAELVKPGASVKISCKASGYTFTDYYINWVKQRPGQGLEWIGKIGPGSGSTYYNEKFKGKATLTADKSSSTAYMQLSSLTSEDSAVYFCARIGSSFFDYWGQGTTLTVSS

SEQ ID NO: 24 - protein, 107 aa, Mus musculus
DIKMTQSPSSMYASLGERVTITCKASQDINSYLSWFQQKPGKSPKTLIYRANRLVDGVPSRFSGSGSGQDYSLTISSLEYEDMGIYYCLQYDEFPLTFGAGTKLELK

SEQ ID NO: 25 - protein, 120 aa, Mus musculus
QVQLLQSGAELVRPGTAVKMSCKASEYTFTNYWIGWARQRPGHGLEWIGDIYPGGGYINYNEKFKGKATLTADKSSSTVYMQFSSLTSEDSAIYYCARGGSNYVGHFDYWGQGTTLTVSS

SEQ ID NO: 26 - protein, 107 aa, Mus musculus
DIQMTQTTSSLSASLGDRVTISCRASQDISNYLNWYQQKPDGTVKLLIYYTSILHSRVPSRFSGSGSGTDYSLTISNLEQEDIATYFCQHGHTLPWTFGGGTKLEIK

SEQ ID NO: 27 - protein, 8 aa, Mus musculus
GYTFISYW

SEQ ID NO: 28 - protein, 8 aa, Mus musculus
IFPSDSET

SEQ ID NO: 29 - protein, 11 aa, Mus musculus
GRRDSSGWIDY

SEQ ID NO: 30 - protein, 6 aa, Mus musculus
QDISNY

SEQ ID NO: 31 - protein, 9 aa, Mus musculus
QQSSMLPFT

SEQ ID NO: 32 - protein, 8 aa, Mus musculus
GYTFTSYW

SEQ ID NO: 33 - protein, 8 aa, Mus musculus
IYPSDGET

SEQ ID NO: 34 - protein, 9 aa, Mus musculus
ARGTTLFDY

SEQ ID NO: 35 - protein, 11 aa, Mus musculus
QSIVHINGNTY

SEQ ID NO: 36 - protein, 9 aa, Mus musculus
FQGSHVPWT

SEQ ID NO: 37 - protein, 8 aa, Mus musculus
GYIFISYW

SEQ ID NO: 38 - protein, 8 aa, Mus musculus
IDPSDSYI

SEQ ID NO: 39 - protein, 14 aa, Mus musculus
ATGDMGDDFYAMDY

SEQ ID NO: 40 - protein, 11 aa, Mus musculus
KSLLYKDGKTY

SEQ ID NO: 41 - protein, 9 aa, Mus musculus
QQLVEYPFT

SEQ ID NO: 42 - protein, 8 aa, Mus musculus
GYTFTTYW

SEQ ID NO: 43 - protein, 8 aa, Mus musculus
IHPSDSDS

SEQ ID NO: 44 - protein, 8 aa, Mus musculus
AIGRGFAY

SEQ ID NO: 45 - protein, 10 aa, Mus musculus
ESVDNYGNSF

SEQ ID NO: 46 - protein, 9 aa, Mus musculus
QQGNEDPYT

SEQ ID NO: 47 - protein, 8 aa, Mus musculus
GYAFTNYL

SEQ ID NO: 48 - protein, 8 aa, Mus musculus
INPGSGGT

SEQ ID NO: 49 - protein, 10 aa, Mus musculus
ARDYGSTFDY

SEQ ID NO: 50 - protein, 6 aa, Mus musculus
QSISSN

SEQ ID NO: 51 - protein, 9 aa, Mus musculus
QQSNSWPLT

SEQ ID NO: 52 - protein, 8 aa, Mus musculus
GYAFTDYL

SEQ ID NO: 53 - protein, 8 aa, Mus musculus
INPGRGGT

SEQ ID NO: 54 - protein, 13 aa, Mus musculus
ARYYGRSFGYFDV

SEQ ID NO: 55 - protein, 6 aa, Mus musculus
QTIGTW

SEQ ID NO: 56 - protein, 9 aa, Mus musculus
QQLYSPPLT

SEQ ID NO: 57 - protein, 8 aa, Mus musculus
GYTFTSYW

SEQ ID NO: 58 - protein, 8 aa, Mus musculus
IYPSDSET

SEQ ID NO: 59 - protein, 11 aa, Mus musculus
TRRDSSGWIDY

SEQ ID NO: 60 - protein, 6 aa, Mus musculus
QDISNY

SEQ ID NO: 61 - protein, 9 aa, Mus musculus
QQGNTLPFT

SEQ ID NO: 62 - protein, 8 aa, Mus musculus
GFSFNTYT

SEQ ID NO: 63 - protein, 10 aa, Mus musculus
IRSKSNNYET

SEQ ID NO: 64 - protein, 11 aa, Mus musculus
VSPDSDSWFAY

SEQ ID NO: 65 - protein, 6 aa, Mus musculus
QNINVW

SEQ ID NO: 66 - protein, 9 aa, Mus musculus
QQGQSYPLT

SEQ ID NO: 67 - protein, 8 aa, Mus musculus
GYTFSTYW

SEQ ID NO: 68 - protein, 8 aa, Mus musculus
IYPGGDST

SEQ ID NO: 69 - protein, 11 aa, Mus musculus
ARGITGGYFDY

SEQ ID NO: 70 - protein, 6 aa, Mus musculus
QDISNY

SEQ ID NO: 71 - protein, 9 aa, Mus musculus
QQGHTLPWT

SEQ ID NO: 72 - protein, 8 aa, Mus musculus
GFSLSSYG

SEQ ID NO: 73 - protein, 7 aa, Mus musculus
IWSGGST

SEQ ID NO: 74 - protein, 12 aa, Mus musculus
VSFNYGSSSFAY

SEQ ID NO: 75 - protein, 6 aa, Mus musculus
QDVRTA

SEQ ID NO: 76 - protein, 9 aa, Mus musculus
QQHYSTPLT

SEQ ID NO: 77 - protein, 8 aa, Mus musculus
GYTFTTYW

SEQ ID NO: 78 - protein, 8 aa, Mus musculus
IDPSDSET

SEQ ID NO: 79 - protein, 12 aa, Mus musculus
ARGDGYYVYFAY

SEQ ID NO: 80 - protein, 7 aa, Mus musculus
SSISSSN

SEQ ID NO: 81 - protein, 9 aa, Mus musculus
QQWSSFPLT

SEQ ID NO: 82 - protein, 8 aa, Mus musculus
GYTFTDYY

SEQ ID NO: 83 - protein, 8 aa, Mus musculus
IGPGSGST

SEQ ID NO: 84 - protein, 10 aa, Mus musculus
ARIGSSFFDY

SEQ ID NO: 85 - protein, 6 aa, Mus musculus
QDINSY

SEQ ID NO: 86 - protein, 9 aa, Mus musculus
LQYDEFPLT

SEQ ID NO: 87 - protein, 8 aa, Mus musculus
EYTFTNYW

SEQ ID NO: 88 - protein, 8 aa, Mus musculus
IYPGGGYI

SEQ ID NO: 89 - protein, 13 aa, Mus musculus
ARGGSNYVGHFDY

SEQ ID NO: 90 - protein, 6 aa, Mus musculus
QDISNY

SEQ ID NO: 91 - protein, 9 aa, Mus musculus
QHGHTLPWT

SEQ ID NO: 92 - DNA, 355 bp, Mus musculus
caggtccaactgcagcagcctggggctgagctggtgaggcctgggtcatcagtgaagctgtcctgcaaggcttctggctacacttttatcagctactggatggattgggtgaagcagaggcctggacaaggccttgaatggattggtaacattttcccttctgatagtgaaactcactacaatcaaaaattcagggacaaggccacattgactgtagacaaatcctccagcacagcctccatacacctcagcagcctgacatctgaggactctgcggtctattactgtggaagaagagacagctcaggctggattgactactggggccaaggcaccactctcacagtctcctcag

SEQ ID NO: 93 - DNA, 322 bp, Mus musculus
gatatccagatgacacagactacatcctccctatctgcctctctgggagacagagtcaccatcagttgcagggcaagtcaggacattagcaattatttaaattggtatcagcagaaaccagatggaactgttaaactcctgatctactacacatcaagattccactcaggagtcccatcaaggttcagtggcagtgggtctggaacagattattctctcaccattcacaatgtggagcaagaagatattgccacttacttttgccaacagagtagtatgcttcctttcacgttcggctcggggacaaagttggaaatgaaac

SEQ ID NO: 94 - DNA, 349 bp, Mus musculus
caggtccaactgcagcagcctggggctgagctggtgaggcctgggtcttcagtgaagttgtcctgcagggcttctggctacaccttcaccagctactggatggattgggtgaagcagaggcctggacaaggccttgaatggattggtaatatttacccttctgatggtgaaactcactacaatcaagacttcaaggacaaggccacattgactgtagacaaatcctccagcacagcctacatgcagctcagcagcctgacatctgaggactctgcggtctattactgtgcaagagggactaccttatttgactattggggccaaggcaccactctcacagtctcctcag

SEQ ID NO: 95 - DNA, 337 bp, Mus musculus
gatgttttgatgacccaaactccactctccctgcctgtcagtcttggagatcaagcctccatctcttgcagatctagtcagagcattgtacatattaatggaaacacctatttagaatggtacctgcagaaaccaggccagtctccaaagctcctgatctacaaagtttccaaccgattttctggggtcccagacaggttcagtggcagtggatcagggacagatttcacactcaagatcagcagagtggaggctgaggatctgggaatttattactgctttcaaggttcacatgttccgtggacgttcggtggaggcaccaagctggaaatcaaac

SEQ ID NO: 96 - DNA, 364 bp, Mus musculus
caggtccaactgcagcagcctggggctgagcttgtgaagcctcgggcttcagttaagctgtcctgcagggcctctggctacatcttcataagttactggatgcagtgggtaaaacagaggcctggacagggccttgagtggatcggagagattgatccttctgatagctatattaactacaatcaaaagttcaagggcaaggcctcattgactgtagacacatcctccaacacagcctacatgcagctcagcagcctgacatctgaggactctgcggtctattactgtgcaacgggcgacatgggggatgatttctatgctatggactactggggtcaaggaacctcagtcaccgtctcctcag

SEQ ID NO: 97 - DNA, 337 bp, Mus musculus
gatattgtgatgaaccaggatgaactctccaatcctgtcacttctggagaatcagtttccatctcctgcaggtctagtaagagtctcctatataaggatgggaagacatacttgaattggtttctgcagagaccaggacaatctcctcagctcctgatctatttgatgtccacccgtgcatcaggagtctcagaccggtttagtggcagtgggtcaggaacagatttcaccctggaaatcagtagagtgaaggctgaggatgtgggtgtgtattactgtcaacaacttgtagagtatccgttcacgttcggaggggggaccaagctggaaataaaac

SEQ ID NO: 98 - DNA, 346 bp, Mus musculus
caggtccaactgcagcagcctggggctgaactggtgaagcctggggcttcagtgaaggtgtcctgcaaggcttctggctacaccttcaccacctactggatgcactgggtgaagcagaggcctggccaaggccttgagtggattggaaggattcatccttctgatagtgatagtaactacaatcaaaagttcaagggcaaggccacattgactgtagacaaatcctccagcacagcctacatgcagctcagcagcctgacatctgaggactctgcggtctattactgtgcaataggcagggggtttgcttactggggccaagggactctggtcactgtctctgcag

SEQ ID NO: 99 - DNA, 334 bp, Mus musculus
gacattgtgctgacccaatctccagcttctttggctgtgtctctaggccagagggccgccatatcctgcagagccagtgaaagtgttgataattatggcaatagttttatgcactggtaccagcagaaaccaggacagccacccaaactcctcatctatcgtgcatccaacctagaatctgggatccctgccaggttcagtggcagtgggtctaggacagacttcaccctcaccattaatcctgtggaggctgatgatgttgcaacctattactgtcagcaaggtaatgaggatccgtacacgttcggaggggggaccaagctggaaataaaac

SEQ ID NO: 100 - DNA, 352 bp, Mus musculus
caggtccagctgcagcagtctggagctgagctggtaaggcctgggacttcagtgaaggtgtcctgcaaggcttctggatacgccttcactaattacttgatagagtgggtaaagcagaggcctggacagggccttgagtggattggagtgattaatcctggaagtggtggtactaactacaatgagaagttcaagggcaaggcaacactgactgcagacaaatcctccagcactgcctacatgcagctcagcagcctgacatctgaggactctgcggtctatttctgtgcaagagactacggtagtacctttgactactggggccaaggcaccactctcacagtctcctcag

SEQ ID NO: 101 - DNA, 322 bp, Mus musculus
gatattgtgctaactcagtctccagccaccctgtctgtgactccaggagatagcgtcagtctttcctgtagggccagccaaagtattagcagcaacctacactggtatcaacaaaaatcacatgagtctccaaggcttctcatcaactttgcttcccagtccatctctgggatcccctccaggttcagtggcagtggatcagggacagatttcactcttaatattaacactgtggagactgaagattttggaatgtatttctgtcaacagagtaacagctggcctctcacgttcggtgctgggaccaagctggagctgaaac

SEQ ID NO: 102 - DNA, 361 bp, Mus musculus
caggtccagctgcagcagtctggagctgagctggtaaggcctgggacttcagtgaaggtgtcctgcaaggcttctggatacgccttcactgattacttgatagagtgggtaaagcagaggcctggacagggccttgagtggattggagtgattaatcctggacgtggtggtactaactacaatgaaaagttcaagggcaaggcaacactgactgcagacaaatcctccagcactgcctacatgcaactcagcagcctgacatctgaggactctgcggtctatttctgtgcaagatactacggtcgtagcttcgggtacttcgatgtctggggcacagggaccacggtcaccgtctcctcag

SEQ ID NO: 103 - DNA, 322 bp, Mus musculus
gacattcagatgacccagtctcctgcctcccagtctgcatctctgggagaaagtgtcaccatcacatgcctggcaagtcagaccattggtacatggttagcatggtatcagcagaaaccagggaaatctcctcagctcctgatttatgctgcaaccagcttggcagatggggtcccatcaaggttcagtggtagtggatctggcacaaaattttctttcaagatcagcagcctacaggctgaagattttgtaagttattactgtcaacaactttacagtcctcctctcacgttcggtgctgggaccaagctggagctgaagc

SEQ ID NO: 104 - DNA, 355 bp, Mus musculus
caggtccaactgcagcagcctggggctgagctggtgaggcctgggtcttcagtgaagctgtcctgcaaggcttctggctacaccttcaccagctactggatggattgggtgaagcagaggcctggacaaggccttgaatggattggtaacatttacccttctgatagtgaaactcactacaatcaaaagttcaaggacagggccacattgactgtagacaaatcctccaccacagcctacatgcagctcagcagcctgacatctgaggactctgcggtctattactgtacaagacgtgacagctcaggctggattgactactggggccaaggcaccactctcacagtctcctcag

SEQ ID NO: 105 - DNA, 322 bp, Mus musculus
gatatccagatgacacagactacatcctccctgtctgcctctctgggagacagagtcaccatcagttgcagggcaagtcaggacattagcaattatttaaactggtatcagcagaaaccagatggaactgttaaactcctgatctactacacatcaagattacactcaggagtcccatcaaggttcagtggccgtgggtctggaacagattattctctcaccattagcaacctggagcaggaagatattgccacttacttttgccaacagggtaatacgcttccattcacgttcggctcggggacacagttggaaataaaac

SEQ ID NO: 106 - DNA, 361 bp, Mus musculus
gaggtgcaacttgttgagtctggtggaggattggtgcagcctaaagggtcattgaaactctcatgtgcagcctctggattcagcttcaatacctacaccatgaactgggtccgccaggctccaggaaagggtttggaatgggttgctcgcataagaagtaaaagtaataattatgaaacatattatgccgattcagtgaaagacagattcaccatctccagagatgattcagaaagcatgctctatctgcaaatgaacaacttgaaaactgaggacacagccatgtattactgtgtgagccccgactctgattcctggtttgcttactggggccaagggactctggtcactgtctctgcag

SEQ ID NO: 107 - DNA, 322 bp, Mus musculus
gacatccagatgaaccagtctccatccagtctgtctgcatcccttggagacacaattaccatcgcttgccatgccagtcagaacattaatgtttggttaagctggtaccagcagaaaccaggaaatattcctaaactattgatctataaggcttccaacttgcacacaggcgtcccatcaaggtttagtggcagtggatctggaacaggtttcacattaaccatcagcagcctgcagcctgaagacattgccacttactactgtcaacagggtcaaagttatcctctgacgttcggtggaggcaccaagctggaaatcaaac

SEQ ID NO: 108 - DNA, 355 bp, Mus musculus
caggtccaactgcagcagcctggggctgagcttgtgaagcctggggcttcagtgaagatgtcctgcaaggcttctggctacaccttcagcacctactggataacctgggtgaagcagaggcctggacaaggccttgagtggattggagatatttatcctggtggtgatagtactaactacaatgagaagttcaagagcaaggccacactgactgaagacacatcctccagcacagtctacatgcagctcagcagcctgacatctgaacactctgcggtctattactgtgcaaggggtattaccgggggctactttgactactggggccaaggcaccactctcacagtgtcctcag

SEQ ID NO: 109 - DNA, 322 bp, Mus musculus
gatatccagatgacacagactacatcctccctgtctgcctctctgggagacagagtcaccatcacttgcagggcaagtcaggacattagcaattatttaaactggtatcagcggaagccagatggaactgttagactcctgatctactacacatcaggattacactcaggagtcccatcaaggttcagtggcagtgggtctggaacagattattctctcaccattagcaacctggagcaagaagattttgccacttacttttgccaacagggtcatacgcttccgtggacgttcggtggaggcaccaacctggaaatcaaac

SEQ ID NO: 110 - DNA, 355 bp, Mus musculus
caggtgcagctgaagcagtcaggacctggcctagtgcagacctcacagagcctgtccatcacctgcacagtctctggtttctcattaagtagttatggtgtacactgggttcgccagtctccaggaaagggtctggagtggctgggagtgatatggagtggtggaagcacagactataatgcagctttcacatccagactgagcatcagcaaggacaattccaagagccaagttttctttaaaatgaacagtctgcaagctgatgacacagccatgtattactgtgtcagctttaactacggtagtagctcgtttgcttactggggccaagggactctggtcactgtctctgcag

SEQ ID NO: 111 - DNA, 322 bp, Mus musculus
gacattgtgatgacccagtctcacaaattcatgtccacatcagtaggagacagggtcagcatcacctgcaaggccagtcaggatgtgaggactgctgtagcctggtatcaacagaaaccaggacaatctcctaaactactgatttactcggcatcctaccggtacactggagtccctgatcgcttcactggcagtggatctgggacggatttcactttcaccatcagcagtgtgcaggctgaagacctggcagtttattattgtcagcaacattatagtactcctctcacgttcggtgctgggaccaagctggagctgaaac

SEQ ID NO: 112 - DNA, 358 bp, Mus musculus
caggtccaactgcagcagcctggggctgagctggtgaggcctgggtcttcagtgaagctgtcctgcaaggcttctggctacaccttcaccacctactggatgcattgggtgaagcagaggcctatacaaggccttgaatggattggtaacattgacccttctgatagtgaaactcactacaatcaaaagttcaaggacaaggccacattgactgtggacaaatcctccagcacagcctacatgcagctcaacagcctgacatctgaggactctgcggtctattactgtgcaagaggggatggttactacgtctactttgcctactggggccaaggcaccactctcacagtctcctcag

SEQ ID NO: 113 - DNA, 325 bp, Mus musculus
gaaattgtgctcacccagtctccagcactcatggctgcatctccaggggagaaggtcaccatcacctgcagtgtcagctcaagtataagttccagcaacttgcactggtaccagcagaagtcagaaacctcccccaaaccctggatttatgccacatccaacctggcttctggagtccctgttcgcttcagtggcagtggatctgggacctcttattctctcacaatcagcagcatggcggctgaagatgctgccacttatttctgtcaacagtggagtagtttcccactcacgttcggtgctgggaccaagctggagctgaaac

SEQ ID NO: 114 - DNA, 352 bp, Mus musculus
caggtccagctgaagcagtctggagctgagctggtgaagcctggggcttcagtgaagatatcctgcaaggcttctggctacaccttcactgactactatataaactgggtgaagcagaggcctggacagggccttgagtggattggaaagattggtcctggaagtggtagtacttactacaatgagaagttcaagggcaaggccacactgactgcagacaaatcctccagcacagcctacatgcagctcagcagcctgacatctgaggactctgcagtctatttctgtgcaagaatcggtagtagtttttttgactactggggccaaggcaccactctcacagtctcctcag

SEQ ID NO: 115 - DNA, 322 bp, Mus musculus
gacatcaagatgacccagtctccatcttccatgtatgcatctctaggagagagagtcactatcacttgcaaggcgagtcaggacattaatagctatttaagctggttccagcagaaaccagggaaatctcctaagaccctgatctatcgtgcaaacagattggtagatggggtcccatcaaggttcagtggcagtggatctgggcaagattattctctcaccatcagcagcctggagtatgaagatatgggaatttattattgtctacagtatgatgagtttcctctcacgttcggtgctgggaccaagctggagctgaaac

SEQ ID NO: 116 - DNA, 361 bp, Mus musculus
caggtccagctgctgcagtctggagctgagctggtaaggcctgggactgcagtgaagatgtcctgcaaggcttctgaatacaccttcactaactactggataggttgggcaaggcagaggcctggacatggccttgagtggattggagatatttaccctggaggtggttatattaactacaatgagaagttcaagggcaaggccacactgactgcagacaaatcctccagcacagtctacatgcagttcagcagcctgacatctgaggactctgccatctattactgtgcaagagggggtagtaactacgtaggacactttgactactggggccaaggcaccactctcacagtctcctcag

SEQ ID NO: 117 - DNA, 322 bp, Mus musculus
gatatccagatgacacagactacatcctccctgtctgcctctctgggagacagagtcaccatcagttgcagggcaagtcaggacattagcaattatttaaactggtatcagcagaagccagatggaactgttaaactcctgatctactacacatcaatattacactctcgagtcccatcaaggttcagtggcagtgggtctggaacagattattctctcaccattagcaacctggagcaagaagatattgccacttacttttgccaacatggtcatacccttccgtggacgttcggtggaggcaccaagctggaaatcaaac

SEQ ID NO: 118 - DNA, 4371 bp, Mus musculus
atgaggcttctcctgcttctggcttttatctctgtcatccctgtctctgttcagctattggacgcgaggcaatttttaatctataatgaagatcacaagcgctgcgtggacgctctaagtgccatctcagttcagacggcaacttgcaacccggaagctgaatcccagaaattccgctgggtgtcagattctcagatcatgagtgttgctttcaaattatgtttgggagtgccatcaaaaactgactgggcttccgtcaccctgtatgcctgtgattcgaaaagtgaatatcagaaatgggagtgtaagaatgacacactctttggaatcaagggcacagagttatattttaattatggcaacagacaagagaagaatatcaagctttacaaaggttcgggattgtggagcagatggaaggtctatggaaccacggatgacctgtgctcgagaggatatgaagccatgtactccttactgggcaatgcaaatggagccgtctgtgcatttccattcaagtttgaaaacaagtggtatgcagactgcacctctgccgggcgctcggacggatggctctggtgtggaaccaccactgactacgacaaagacaagctgtttggattttgtccattgcactttgagggaagcgagagattatggaacaaagatccactgactggcattctttaccagataaactccaagtctgctttaacctggcatcaggcaagggcaagctgcaagcagcagaatgctgacctcctgagtgtcacggagatccacgagcaaatgtacctcacaggattaaccagttccttgagctcgggactctggattggactcaacagtctgagtgtacgcagtggttggcagtgggctggaggaagcccattccggtatctgaactggctaccaggaagtccatcatcagagcctggaaagagctgtgtgtcactaaaccctggaaaaaatgccaagtgggaaaatctggaatgtgttcagaagcttggctacatttgtaaaaagggaaacaataccttgaacccatttatcattccctcagcaagcgatgtgcctaccggctgccctaatcagtggtggccctatgcaggccactgctacaggatccatagggaagagaagaagatccagaaatatgctttgcaagcttgtaggaaggagggtggggacctggcaagtatccacagcattgaggagtttgacttcatcttctcccagctcggatatgagccaaatgatgagctgtggattggtttaaatgacatcaagattcagatgtactttgagtggagtgatggaaccccagtgacatttactaaatggcttcctggagagccaagccatgagaacaacagacaggaggactgcgtggttatgaaaggcaaggatggatactgggcggacagagcctgtgagcaaccactaggttacatctgtaagatggtatcacaaagccatgctgtagtaccggagggtgcagacaaaggctgccggaaaggctggaaacggcatgggttttactgctacttgattggatccactctatccaccttcactgatgcaaaccacacatgcacaaatgaaaaggcttatttaacaacagttgaagacagatatgaacaagcattcctgactagtttggttggattgaggcctgaaaaatatttttggacaggactctcagatgttcaaaacaaagggacgtttcggtggactgtggacgagcaggtgcagtttacacactggaatgccgacatgccaggacgaaaggcgggatgtgttgccatgaaaaccggagtggcaggtggcttatgggatgttttgagttgtgaagaaaaggcaaaatttgtgtgcaaacattgggcagaaggagtgactcgcccaccagagcccacaacaactcctgaacccaaatgtccagaaaactggggtaccaccagtaaaaccagcatgtgtttcaaactgtatgcaaaaggaaagcatgaaaagaaaacgtggtttgaatctcgagatttttgcaaagctataggtggagagctggcgagcatcaagagtaaagatgaacagcaagtgatttggaggctgattacgagcagtggaagctaccatgagctgttttggttgggactgacctatggaagtccttcagaggggttcacctggagtgatggttctcccgtttcctatgaaaattgggcttacggtgaaccaaataattaccaaaatgttgaatattgtggtgagctgaaaggtgaccctggcatgtcctggaatgatatcaactgtgaacacctcaacaactggatttgtcagatacaaaaagggaaaacactactacctgagcccacacctgctccacaagacaatccaccagttactgcagatgggtgggttatttacaaagactaccagtactattttagcaaagagaaggaaaccatggacaacgcgcgagcattttgcaagaagaattttggtgatcttgctacaattaaaagtgaaagtgaaaagaagtttctatggaaatatataaacaagaatggtgggcagtcaccatattttattggcatgttaatcagcatggataagaaattcatttggatggatgggagcaaagtagattttgtggcttgggctacaggagaacccaactttgcaaatgatgatgaaaactgtgtaacgatgtacacaaattcagggttctggaatgacatcaactgtggttatccaaataacttcatctgccagagacataacagcagcatcaatgccactgccatgcctaccacacccacgacaccaggtggctgcaaggaaggttggcatttgtacaagaacaagtgctttaaaatttttggatttgctaatgaagaaaaaaaaagctggcaagacgcacggcaagcttgcaaaggactgaaaggaaacctggtgtccatagaaaatgcacaagagcaagcatttgttacctatcacatgagagactccactttcaatgcctggactgggctgaatgatatcaacgcagaacacatgttcctgtggacagctggacaaggagttcattatacaaactgggggaaaggctatcctggtggaagaagaagtagcctatcttatgaagatgctgactgtgtagttgtgattggtggcaattcacgagaggcagggacctggatggatgacacctgtgacagtaaacaaggctatatatgtcaaacacagactgacccttccctgcctgtttctccaaccactactccaaaagatggctttgttacatatgggaaaagcagctattcccttatgaaattgaagctaccatggcatgaagcagagacatattgcaaggatcatacttccctgcttgctagcattctagacccctacagtaatgcatttgcatggatgaaaatgcacccatttaatgtacccatatggattgccctgaacagcaacttgaccaataatgaatatacttggacggatagatggagggtgcggtacactaactggggtgctgacgagccgaagcttaagtcagcatgtgtttacatggatgttgatggctactggagaacatcatactgcaatgaaagtttttattttctctgcaaaaaatcagacgaaatccctgctactgaacctcctcaactgcctggcaagtgtccagagtcagaacagactgcgtggattcctttctatggccattgctactattttgaatcttcttttacgagaagttggggtcaggcttctctggaatgccttcgaatgggtgcctccctggtttccatcgagactgctgctgagtccagttttctgtcataccgtgttgaacctcttaaaagtaaaaccaatttttggataggcatgttccgaaatgttgaagggaagtggctttggttgaacgacaatcctgtctcctttgtcaactggaaaacaggcgatccctctggtgaacggaatgattgtgtagttctagcttcatcttcgggcctttggaataatatccactgttcttcgtacaaaggatttatttgtaaaatgccaaaaattattgatcctgtaactacacactcatccattacaaccaaagctgaccaaaggaagatggatcctcaacccaagggctcttctaaagcagcaggagtggtcaccgtggtcctcctgattgtgataggtgccggcgttgcagcctatttcttttataagaaaaggcatgcgttgcacatacctcaagaggccacctttgaaaacactctctacttcaacagtaatctgagtccaggaacaagtgacacgaaagatctcatgggcaacatcgagcagaatgagcatgcgatcatttag